European Patent Application EP 4 299 591 A1, published January 3, 2024. Title: Preparation of Siglec-15 Binding Protein and Use Thereof. Applicant: SHANGHAI JEMINCARE PHARMACEUTICAL CO., LTD.; JIANGXI JEMINCARE GROUP CO., LTD. The sequence listing filed with the application follows.

SEQUENCE LISTING (41 sequences)

SEQ ID NO: 1 - protein, 13 aa, Artificial Sequence
  HCDR3 0+2+3+5+6+7+9+13+15
AIGSSWYSDAFDL

SEQ ID NO: 2 - protein, 6 aa, Artificial Sequence
  HCDR2 0+2+9
SGGGGS

SEQ ID NO: 3 - protein, 6 aa, Artificial Sequence
  HCDR2 3+13+15
TGGGES

SEQ ID NO: 4 - protein, 6 aa, Artificial Sequence
  HCDR2 5
YGGGGS

SEQ ID NO: 5 - protein, 6 aa, Artificial Sequence
  HCDR2 6
WGGGGS

SEQ ID NO: 6 - protein, 6 aa, Artificial Sequence
  HCDR2 7
SGGGVY

SEQ ID NO: 7 - protein, 7 aa, Artificial Sequence
  HCDR1 0+3+5+6+7+9+13+15
GFTFSSY

SEQ ID NO: 8 - protein, 7 aa, Artificial Sequence
  HCDR1 2
GFTSSSY

SEQ ID NO: 9 - protein, 9 aa, Artificial Sequence
  LCDR3 0+2+3+5+6+7+9+13+15
QQSYSIPYT

SEQ ID NO: 10 - protein, 7 aa, Artificial Sequence
  LCDR2 0+2+3+5+6+7+9
VASSLQS

SEQ ID NO: 11 - protein, 7 aa, Artificial Sequence
  LCDR2 13
VASFEHR

SEQ ID NO: 12 - protein, 7 aa, Artificial Sequence
  LCDR2 15
VASYIHS

SEQ ID NO: 13 - protein, 11 aa, Artificial Sequence
  LCDR1 0+2+3+5+6+7+13+15
RASQDISSWLA

SEQ ID NO: 14 - protein, 11 aa, Artificial Sequence
  LCDR1 9
RASQDISDWLA

SEQ ID NO: 15 - protein, 25 aa, Artificial Sequence
  HFR1
EVQLLESGGGLVQPGGSLRLSCAAS

SEQ ID NO: 16 - protein, 19 aa, Artificial Sequence
  HFR2
AMSWVRQAPGKGLEWVSTI

SEQ ID NO: 17 - protein, 41 aa, Artificial Sequence
  HFR3
TYYADSVKGRFTISRDNSKNTLYLQMNSLRAEDTAVYYCAK

SEQ ID NO: 18 - protein, 11 aa, Artificial Sequence
  HFR4
WGQGTMVTVSS

SEQ ID NO: 19 - protein, 23 aa, Artificial Sequence
  LFR1
DIQMTQSPSSVSASVGDRVTITC

SEQ ID NO: 20 - protein, 15 aa, Artificial Sequence
  LFR2
WYQQKPGKAPKLLIY

SEQ ID NO: 21 - protein, 32 aa, Artificial Sequence
  LFR3
GVPSRFSGSGSGTDFTLTISSLQPEDFATYYC

SEQ ID NO: 22 - protein, 10 aa, Artificial Sequence
  LFR4
FGQGTKLEIK

SEQ ID NO: 23 - protein, 122 aa, Artificial Sequence
  VH 0+9
EVQLLESGGGLVQPGGSLRLSCAASGFTFSSYAMSWVRQAPGKGLEWVSTISGGGGSTYYADSVKGRFTISRDNSKNTLYLQMNSLRAEDTAVYYCAKAIGSSWYSDAFDLWGQGTMVTVSS

SEQ ID NO: 24 - protein, 122 aa, Artificial Sequence
  VH 2
EVQLLESGGGLVQPGGSLRLSCAASGFTSSSYAMSWVRQAPGKGLEWVSTISGGGGSTYYADSVKGRFTISRDNSKNTLYLQMNSLRAEDTAVYYCAKAIGSSWYSDAFDLWGQGTMVTVSS

SEQ ID NO: 25 - protein, 122 aa, Artificial Sequence
  VH 3+13+15
EVQLLESGGGLVQPGGSLRLSCAASGFTFSSYAMSWVRQAPGKGLEWVSTITGGGESTYYADSVKGRFTISRDNSKNTLYLQMNSLRAEDTAVYYCAKAIGSSWYSDAFDLWGQGTMVTVSS

SEQ ID NO: 26 - protein, 122 aa, Artificial Sequence
  VH 5
EVQLLESGGGLVQPGGSLRLSCAASGFTFSSYAMSWVRQAPGKGLEWVSTIYGGGGSTYYADSVKGRFTISRDNSKNTLYLQMNSLRAEDTAVYYCAKAIGSSWYSDAFDLWGQGTMVTVSS

SEQ ID NO: 27 - protein, 122 aa, Artificial Sequence
  VH 6
EVQLLESGGGLVQPGGSLRLSCAASGFTFSSYAMSWVRQAPGKGLEWVSTIWGGGGSTYYADSVKGRFTISRDNSKNTLYLQMNSLRAEDTAVYYCAKAIGSSWYSDAFDLWGQGTMVTVSS

SEQ ID NO: 28 - protein, 122 aa, Artificial Sequence
  VH 7
EVQLLESGGGLVQPGGSLRLSCAASGFTFSSYAMSWVRQAPGKGLEWVSTISGGGVYTYYADSVKGRFTISRDNSKNTLYLQMNSLRAEDTAVYYCAKAIGSSWYSDAFDLWGQGTMVTVSS

SEQ ID NO: 29 - protein, 107 aa, Artificial Sequence
  VL 0+2+3+5+7
DIQMTQSPSSVSASVGDRVTITCRASQDISSWLAWYQQKPGKAPKLLIYVASSLQSGVPSRFSGSGSGTDFTLTISSLQPEDFATYYCQQSYSIPYTFGQGTKLEIK

SEQ ID NO: 30 - protein, 107 aa, Artificial Sequence
  VL 9
DIQMTQSPSSVSASVGDRVTITCRASQDISDWLAWYQQKPGKAPKLLIYVASSLQSGVPSRFSGSGSGTDFTLTISSLQPEDFATYYCQQSYSIPYTFGQGTKLEIK

SEQ ID NO: 31 - protein, 107 aa, Artificial Sequence
  VL 13
DIQMTQSPSSVSASVGDRVTITCRASQDISSWLAWYQQKPGKAPKLLIYVASFEHRGVPSRFSGSGSGTDFTLTISSLQPEDFATYYCQQSYSIPYTFGQGTKLEIK

SEQ ID NO: 32 - protein, 107 aa, Artificial Sequence
  VL 15
DIQMTQSPSSVSASVGDRVTITCRASQDISSWLAWYQQKPGKAPKLLIYVASYIHSGVPSRFSGSGSGTDFTLTISSLQPEDFATYYCQQSYSIPYTFGQGTKLEIK

SEQ ID NO: 33 - protein, 6 aa, Artificial Sequence
  HCDR2 formula
  misc_feature (1)..(1): Xaa = Ser, Thr, Trp or Tyr
  misc_feature (5)..(5): Xaa = Glu, Gly or Val
  misc_feature (6)..(6): Xaa = Ser or Tyr
XGGGXX

SEQ ID NO: 34 - protein, 7 aa, Artificial Sequence
  HCDR1 formula
  misc_feature (4)..(4): Xaa = Phe or Ser
GFTXSSY

SEQ ID NO: 35 - protein, 7 aa, Artificial Sequence
  LCDR2 formula
  misc_feature (4)..(4): Xaa = Phe, Ser or Tyr
  misc_feature (5)..(5): Xaa = Glu, Ile or Leu
  misc_feature (6)..(6): Xaa = His or Gln
  misc_feature (7)..(7): Xaa = Arg or Ser
VASXXXX

SEQ ID NO: 36 - protein, 11 aa, Artificial Sequence
  LCDR1 formula
  misc_feature (8)..(8): Xaa = Asp or Ser
RASQDISXWLA

SEQ ID NO: 37 - protein, 122 aa, Artificial Sequence
  VH formula
  misc_feature (29)..(29): Xaa = Phe or Ser
  misc_feature (52)..(52): Xaa = Ser, Thr, Trp or Tyr
  misc_feature (56)..(56): Xaa = Glu, Gly or Val
  misc_feature (57)..(57): Xaa = Ser or Tyr
EVQLLESGGGLVQPGGSLRLSCAASGFTXSSYAMSWVRQAPGKGLEWVSTIXGGGXXTYYADSVKGRFTISRDNSKNTLYLQMNSLRAEDTAVYYCAKAIGSSWYSDAFDLWGQGTMVTVSS

SEQ ID NO: 38 - protein, 107 aa, Artificial Sequence
  VL formula
  misc_feature (31)..(31): Xaa = Asp or Ser
  misc_feature (53)..(53): Xaa = Phe, Ser or Tyr
  misc_feature (54)..(54): Xaa = Glu, Ile or Leu
  misc_feature (55)..(55): Xaa = His or Gln
  misc_feature (56)..(56): Xaa = Arg or Ser
DIQMTQSPSSVSASVGDRVTITCRASQDISXWLAWYQQKPGKAPKLLIYVASXXXXGVPSRFSGSGSGTDFTLTISSLQPEDFATYYCQQSYSIPYTFGQGTKLEIK

SEQ ID NO: 39 - protein, 330 aa, Artificial Sequence
  Heavy chain constant region
ASTKGPSVFPLAPSSKSTSGGTAALGCLVKDYFPEPVTVSWNSGALTSGVHTFPAVLQSSGLYSLSSVVTVPSSSLGTQTYICNVNHKPSNTKVDKKVEPKSCDKTHTCPPCPAPELLGGPSVFLFPPKPKDTLMISRTPEVTCVVVDVSHEDPEVKFNWYVDGVEVHNAKTKPREEQYNSTYRVVSVLTVLHQDWLNGKEYKCKVSNKALPAPIEKTISKAKGQPREPQVYTLPPSREEMTKNQVSLTCLVKGFYPSDIAVEWESNGQPENNYKTTPPVLDSDGSFFLYSKLTVDKSRWQQGNVFSCSVMHEALHNHYTQKSLSLSPGK

SEQ ID NO: 40 - protein, 107 aa, Artificial Sequence [sequence omitted]

SEQ ID NO: 41 - protein, 21 aa, Artificial Sequence
  T2A
GSGEGRGSLLTCGDVEENPGP